European Patent Specification EP 3 677 683 B1, published July 17, 2024. Title: Mutated tetraprenyl- beta-curcumene cyclase and one enzyme method for preparing ambrein using the same. Applicant: NIIGATA UNIVERSITY ADEKA CORPORATION. The sequence listing filed with the application follows.

SEQUENCE LISTING (14 sequences)

SEQ ID NO: 1 - protein, 625 aa, Bacillus megaterium
MIILLKEVQLEIQRRIAYLRPTQKNDGSFRYCFETGVMPDAFLIMLLRTFDLDKEVLIKQLTERIVSLQNEDGLWTLFDDEEHNLSATIQAYTALLYSGYYQKNDRILRKAERYIIDSGGISRAHFLTRWMLSVNGLYEWPKLFYLPLSLLLVPTYVPLNFYELSTYARIHFVPMMVAGNKKFSLTSRHTPSLSHLDVREQKQESEETTQESRASIFLVDHLKQLASLPSYIHKLGYQAAERYMLERIEKDGTLYSYATSTFFMIYGLLALGYKKDSFVIQKAIDGICSLLSTCSGHVHVENSTSTVWDTALLSYALQEAGVPQQDPMIKGTTRYLKKRQHTKLGDWQFHNPNTAPGGWGFSDINTNNPDLDDTSAAIRALSRRAQTDTDYLESWQRGINWLLSMQNKDGGFAAFEKNTDSILFTYLPLENAKDAATDPATADLTGRVLECLGNFAGMNKSHPSIKAAVKWLFDHQLDNGSWYGRWGVCYIYGTWAAITGLRAVGVSASDPRIIKAINWLKSIQQEDGGFGESCYSASLKKYVPLSFSTPSQTAWALDALMTICPLKDQSVEKGIKFLLNPNLTEQQTHYPTGIGLPGQFYIQYHSYNDIFPLLALAHYAKKHSS

SEQ ID NO: 2 - protein, 632 aa, Bacillus subtilis
MGTLQEKVRRYQKKTIAELKNRQNADGSWTFCFEGPIMTNSFFILLLTSLDEGENEKELISALAAGIREKQQPDGTFINYPDETSGNITATVQGYVGMLASGCFHRSDPHMRKAEQSIISHGGLRHVHFMTKWMLAVNGLYPWPVLYLPLSLMALPPTLPVHFYQFSAYARIHFAPMAVTLNQRFVLKNRNIPSLRHLDPHMTKNPFTWLRSDAFEERDLTSIWSHWNRIFHAPFAFQQLGLQTAKTYMLDRIEKDGTLYSYASATIFMVYSLLSLGVSRYSPVIKRAINGIKSLMTKCNGIPYLENSTSTVWDTALISYALQKNGVTETDGSITKAAAYLLERQHTKRADWSVKNPSAAPGGWGFSNINTNNPDCDDTAAVLKAIPHSYSPSAWERGVSWLLSMQNNDGGFSAFEKNVNHPLIRLLPLESAEDAAVDPSTADLTGRVLHFLGEKAGFTEKHQHIQRAVNWLFEHQEQNGSWYGRWGVCYIYGTWAALTGMHACEVDRKHPAIQKALRWLKSIQHDDGSWGESCNSAEVKTYVPLHKGTIVQTAWALDALLTYESSEHPSVVKGMQYLTDSSYHGADSLAYPAGIGLPKQFYIRYHSYPYVFSLLAVGKYLNSIEKETANET

SEQ ID NO: 3 - protein, 592 aa, Bacillus licheniformis
MTDSFFILMLTSLGDQDSSLIASLAERIRSRQSEDGAFRNHPDERAGNLTATVQGYTGMLASGLYDRKAPHMQKAEAFIKDAGGLKGVHFMTKWMLAANGLYPWPRAYIPLSFLLIPSYFPLHFYHFSTYARIHFVPMAITFNRRFSLKNNQIGSLRHLDEAMSKNPLEWLNIRAFDERTFYSFNLQWKQLFQWPAYVHQLGFEAGKKYMLDRIEEDGTLYSYASATMFMIYSLLAMGISKNAPVVKKAVSGIKSLISSCGKEGAHLENSTSTVWDTALISYAMQESGVPEQHSSTSSAADYLLKRQHVKKADWAVSNPQAVPGGWGFSHINTNNPDLDDTAAALKAIPFQRRPDAWNRGLAWLLSMQNKDGGFAAFEKDVDHPLIRNLPLESAAEAAVDPSTADLTGRVLHLLGLKGRFTDNHPAVRRALRWLDHHQKADGSWYGRWGVCFIYGTWAALTGMKAVGVSANQTSVKKAISWLKSIQREDGSWGESCKSCEAKRFVPLHFGTVVQSSWALEALLQYERPDDPQIIKGIRFLIDEHESSRERLEYPTGIGLPNQFYIRYHSYPFVFSLLASSAFIKKAEMRETY

SEQ ID NO: 4 - protein, 631 aa, Alicyclobacillus acidocaldarius [sequence omitted]

SEQ ID NO: 5 - protein, 625 aa, Bacillus megaterium
MIILLKEVQLEIQRRIAYLRPTQKNDGSFRYCFETGVMPDAFLIMLLRTFDLDKEVLIKQLTERIVSLQNEDGLWTLFDDEEHNLSATIQAYTALLYSGYYQKNDRILRKAERYIIDSGGISRAHFLTRWMLSVNGLYEWPKLFYLPLSLLLVPTYVPLNFYELSTAARIHFVPMMVAGNKKFSLTSRHTPSLSHLDVREQKQESEETTQESRASIFLVDHLKQLASLPSYIHKLGYQAAERYMLERIEKDGTLYSYATSTFFMIYGLLALGYKKDSFVIQKAIDGICSLLSTCSGHVHVENSTSTVWDTALLSYALQEAGVPQQDPMIKGTTRYLKKRQHTKLGDWQFHNPNTAPGGWGFSDINTNNPDLDCTSAAIRALSRRAQTDTDYLESWQRGINWLLSMQNKDGGFAAFEKNTDSILFTYLPLENAKDAATDPATADLTGRVLECLGNFAGMNKSHPSIKAAVKWLFDHQLDNGSWYGRWGVCYIYGTWAAITGLRAVGVSASDPRIIKAINWLKSIQQEDGGFGESCYSASLKKYVPLSFSTPSQTAWALDALMTICPLKDQSVEKGIKFLLNPNLTEQQTHYPTGIGLPGQFYIQYHSYNDIFPLLALAHYAKKHSS

SEQ ID NO: 6 - protein, 625 aa, Bacillus megaterium
MIILLKEVQLEIQRRIAYLRPTQKNDGSFRYCFETGVMPDAFLIMLLRTFDLDKEVLIKQLTERIVSLQNEDGLWTLFDDEEHNLSATIQAYTALLYSGYYQKNDRILRKAERYIIDSGGISRAHFLTRWMLSVNGLYEWPKLFYLPLSLLLVPTYVPLNFYELSTYARIHFVPMMVAGNKKFSLTSRHTPSLSHLDVREQKQESEETTQESRASIFLVDHLKQLASLPSYIHKLGYQAAERYMLERIEKDGTLYSYATSTFFMIYGLLALGYKKDSFVIQKAIDGICSLLSTCSGHVHVENSTSTVWDTALLSYALQEAGVPQQDPMIKGTTRYLKKRQHTKLGDWQFHNPNTAPGGWGFSDINTNNPDLDCTSAAIRALSRRAQTDTDYLESWQRGINWLLSMQNKDGGFAAFEKNTDSILFTYLPLENAKDAATDPATADLTGRVLECLGNFAGMNKSHPSIKAAVKWLFDHQLDNGSWYGRWGVCYIYGTWAAITGLRAVGVSASDPRIIKAINWLKSIQQEDGGFGESCYSASLKKYVPLSFSTPSQTAWALDALMTICPLKDQSVEKGIKFLLNPNLTEQQTHYPTGIGAPGQFYIQYHSYNDIFPLLALAHYAKKHSS

SEQ ID NO: 7 - DNA, 1878 bp, Bacillus megaterium
gtgattattctgctgaaagaggttcagctggagatccagcgtcgcatcgcctatttacgcccgacccagaaaaatgacggcagtttccgctactgcttcgagaccggcgtgatgccggacgcctttctgattatgctgctgcgtaccttcgacctggacaaagaagttctgattaagcagttaaccgagcgcattgtgagcctgcagaacgaagatggtctgtggacactgtttgacgatgaggagcacaacctgagtgccacaatccaggcctataccgccctgctgtacagcggctattaccagaaaaatgaccgcatcttacgtaaggccgaacgctacattatcgatagcggcggcatcagccgtgcacatttcctgacccgttggatgctgagcgttaatggcctgtacgaatggccgaagctgttctacctgccgttaagcctgctgctggttccgacctacgtgccgctgaacttttatgagctgagcaccgcagcccgtattcactttgttccgatgatggtggccggtaataaaaaattcagcttaaccagccgccatacccctagtctgagccacctggatgtgcgtgaacaaaaacaggagagtgaagaaaccacccaggagagccgcgcaagcatcttcttagtggatcatctgaaacagctggccagcctgccgagttacattcataagctgggctaccaggcagcagaacgctatatgctggaacgcatcgaaaaggacggcacactgtacagttacgccaccagcaccttttttatgatttacggcctgctggccctgggctacaaaaaggatagctttgtgattcagaaagcaattgatggcatttgtagtctgctgagtacatgcagcggtcacgtgcacgttgaaaacagtaccagcaccgtttgggacaccgcactgctgagctatgccctgcaagaagcaggcgtgccgcagcaggacccgatgattaagggtaccacccgttatctgaagaaacgccagcatacaaaactgggcgactggcagtttcacaatccgaacaccgcaccgggcggttggggctttagcgacattaacaccaacaatcctgatctggattgcaccagcgccgcaattcgtgcattaagccgccgcgcccagaccgacacagattacctggaaagctggcagcgcggcatcaattggctgctgagcatgcagaacaaggacggcggctttgccgcatttgaaaagaacaccgatagtatcctgttcacctacctgcctctggaaaatgcaaaggatgccgcaaccgatccggccaccgccgatttaaccggccgcgttttagaatgcctgggtaacttcgccggcatgaacaaaagccatccgagcattaaagccgccgtgaaatggctgttcgaccaccagctggataacggtagctggtacggtcgttggggcgtgtgctatatttacggcacctgggccgcaatcacaggtctgcgcgccgtgggtgttagtgccagcgatccgcgtatcatcaaggcaatcaactggctgaaaagcattcagcaagaagatggtggctttggcgaaagctgctacagcgccagcctgaaaaagtatgttccgctgagtttcagcaccccgagtcagacagcctgggcactggacgccctgatgaccatttgcccgttaaaggatcagagcgttgaaaagggcattaaattcctgctgaatccgaacctgacagagcaacagacacactatccgacaggcattggtctgccgggccagttctatattcagtaccacagctacaatgatatctttcctttactggccctggcccactacgcaaaaaagcatagtagctaa

SEQ ID NO: 8 - DNA, 1878 bp, Bacillus megaterium
gtgattattctgctgaaagaggttcagctggagatccagcgtcgcatcgcctatttacgcccgacccagaaaaatgacggcagtttccgctactgcttcgagaccggcgtgatgccggacgcctttctgattatgctgctgcgtaccttcgacctggacaaagaagttctgattaagcagttaaccgagcgcattgtgagcctgcagaacgaagatggtctgtggacactgtttgacgatgaggagcacaacctgagtgccacaatccaggcctataccgccctgctgtacagcggctattaccagaaaaatgaccgcatcttacgtaaggccgaacgctacattatcgatagcggcggcatcagccgtgcacatttcctgacccgttggatgctgagcgttaatggcctgtacgaatggccgaagctgttctacctgccgttaagcctgctgctggttccgacctacgtgccgctgaacttttatgagctgagcacctatgcccgtattcactttgttccgatgatggtggccggtaataaaaaattcagcttaaccagccgccatacccctagtctgagccacctggatgtgcgtgaacaaaaacaggagagtgaagaaaccacccaggagagccgcgcaagcatcttcttagtggatcatctgaaacagctggccagcctgccgagttacattcataagctgggctaccaggcagcagaacgctatatgctggaacgcatcgaaaaggacggcacactgtacagttacgccaccagcaccttttttatgatttacggcctgctggccctgggctacaaaaaggatagctttgtgattcagaaagcaattgatggcatttgtagtctgctgagtacatgcagcggtcacgtgcacgttgaaaacagtaccagcaccgtttgggacaccgcactgctgagctatgccctgcaagaagcaggcgtgccgcagcaggacccgatgattaagggtaccacccgttatctgaagaaacgccagcatacaaaactgggcgactggcagtttcacaatccgaacaccgcaccgggcggttggggctttagcgacattaacaccaacaatcctgatctggattgtaccagcgccgcaattcgtgcattaagccgccgcgcccagaccgacacagattacctggaaagctggcagcgcggcatcaattggctgctgagcatgcagaacaaggacggcggctttgccgcatttgaaaagaacaccgatagtatcctgttcacctacctgcctctggaaaatgcaaaggatgccgcaaccgatccggccaccgccgatttaaccggccgcgttttagaatgcctgggtaacttcgccggcatgaacaaaagccatccgagcattaaagccgccgtgaaatggctgttcgaccaccagctggataacggtagctggtacggtcgttggggcgtgtgctatatttacggcacctgggccgcaatcacaggtctgcgcgccgtgggtgttagtgccagcgatccgcgtatcatcaaggcaatcaactggctgaaaagcattcagcaagaagatggtggctttggcgaaagctgctacagcgccagcctgaaaaagtatgttccgctgagtttcagcaccccgagtcagacagcctgggcactggacgccctgatgaccatttgcccgttaaaggatcagagcgttgaaaagggcattaaattcctgctgaatccgaacctgacagagcaacagacacactatccgacaggcattggtgcaccgggccagttctatattcagtaccacagctacaatgatatctttcctttactggccctggcccactacgcaaaaaagcatagtagctaa

SEQ ID NO: 9 - protein, 625 aa, Bacillus megaterium
MIILLKEVQLEIQRRIAYLRPTQKNDGSFRYCFETGVMPDAFLIMLLRTFDLDKEVLIKQLTERIVSLQNEDGLWTLFDDEEHNLSATIQAYTALLYSGYYQKNDRILRKAERYIIDSGGISRAHFLTRWMLSVNGLYEWPKLFYLPLSLLLVPTYVPLNFYELSTYARIHFVPMMVAGNKKFSLTSRHTPSLSHLDVREQKQESEETTQESRASIFLVDHLKQLASLPSYIHKLGYQAAERYMLERIEKDGTLYSYATSTFFMIYGLLALGYKKDSFVIQKAIDGICSLLSTCSGHVHVENSTSTVWDTALLSYALQEAGVPQQDPMIKGTTRYLKKRQHTKLGDWQFHNPNTAPGGWGFSDINTNNPDLDDTSAAIRALSRRAQTDTDYLESWQRGINWLLSMQNKDGGFAAFEKNTDSILFTYLPLENAKDAATDPATADLTGRVLECLGNFAGMNKSHPSIKAAVKWLFDHQLDNGSWYGRWGVCYIYGTWAAITGLRAVGVSASDPRIIKAINWLKSIQQEDGGFGESCYSASLKKYVPLSFSTPSQTAWALDALMTICPLKDQSVEKGIKFLLNPNLTEQQTHYPTGIGAPGQFYIQYHSYNDIFPLLALAHYAKKHSS

SEQ ID NO: 10 - protein, 625 aa, Bacillus megaterium
MIILLKEVQLEIQRRIAYLRPTQKNDGSFRYCFETGVMPDAFLIMLLRTFDLDKEVLIKQLTERIVSLQNEDGLWTLFDDEEHNLSATIQAYTALLYSGYYQKNDRILRKAERYIIDSGGISRAHFLTRWMLSVNGLYEWPKLFYLPLSLLLVPTYVPLNFYELSTYARIHFVPMMVAGNKKFSLTSRHTPSLSHLDVREQKQESEETTQESRASIFLVDHLKQLASLPSYIHKLGYQAAERYMLERIEKDGTLYSYATSTFFMIYGLLALGYKKDSFVIQKAIDGICSLLSTCSGHVHVENSTSTVWDTALLSYALQEAGVPQQDPMIKGTTRYLKKRQHTKLGDWQFHNPNTAPGGWGFSDINTNNPDLDDTSAAIRALSRRAQTDTDYLESWQRGINWLLSMQNKDGGFAAFEKNTDSILFTYLPLENAKDAATDPATADLTGRVLECLGNFAGMNKSHPSIKAAVKWLFDHQLDNGSWYGRWGVCYIYGTWAAITGLRAVGVSASDPRIIKAINWLKSIQQEDGGFGESCYSASLKKYVPLSFSTPSQTAWALDALMTICPLKDQSVEKGIKFLLNPNLTEQQTHYPTGIGFPGQFYIQYHSYNDIFPLLALAHYAKKHSS

SEQ ID NO: 11 - DNA, 1878 bp, Bacillus megaterium
gtgattattctgctgaaagaggttcagctggagatccagcgtcgcatcgcctatttacgcccgacccagaaaaatgacggcagtttccgctactgcttcgagaccggcgtgatgccggacgcctttctgattatgctgctgcgtaccttcgacctggacaaagaagttctgattaagcagttaaccgagcgcattgtgagcctgcagaacgaagatggtctgtggacactgtttgacgatgaggagcacaacctgagtgccacaatccaggcctataccgccctgctgtacagcggctattaccagaaaaatgaccgcatcttacgtaaggccgaacgctacattatcgatagcggcggcatcagccgtgcacatttcctgacccgttggatgctgagcgttaatggcctgtacgaatggccgaagctgttctacctgccgttaagcctgctgctggttccgacctacgtgccgctgaacttttatgagctgagcacctatgcccgtattcactttgttccgatgatggtggccggtaataaaaaattcagcttaaccagccgccatacccctagtctgagccacctggatgtgcgtgaacaaaaacaggagagtgaagaaaccacccaggagagccgcgcaagcatcttcttagtggatcatctgaaacagctggccagcctgccgagttacattcataagctgggctaccaggcagcagaacgctatatgctggaacgcatcgaaaaggacggcacactgtacagttacgccaccagcaccttttttatgatttacggcctgctggccctgggctacaaaaaggatagctttgtgattcagaaagcaattgatggcatttgtagtctgctgagtacatgcagcggtcacgtgcacgttgaaaacagtaccagcaccgtttgggacaccgcactgctgagctatgccctgcaagaagcaggcgtgccgcagcaggacccgatgattaagggtaccacccgttatctgaagaaacgccagcatacaaaactgggcgactggcagtttcacaatccgaacaccgcaccgggcggttggggctttagcgacattaacaccaacaatcctgatctggatgataccagcgccgcaattcgtgcattaagccgccgcgcccagaccgacacagattacctggaaagctggcagcgcggcatcaattggctgctgagcatgcagaacaaggacggcggctttgccgcatttgaaaagaacaccgatagtatcctgttcacctacctgcctctggaaaatgcaaaggatgccgcaaccgatccggccaccgccgatttaaccggccgcgttttagaatgcctgggtaacttcgccggcatgaacaaaagccatccgagcattaaagccgccgtgaaatggctgttcgaccaccagctggataacggtagctggtacggtcgttggggcgtgtgctatatttacggcacctgggccgcaatcacaggtctgcgcgccgtgggtgttagtgccagcgatccgcgtatcatcaaggcaatcaactggctgaaaagcattcagcaagaagatggtggctttggcgaaagctgctacagcgccagcctgaaaaagtatgttccgctgagtttcagcaccccgagtcagacagcctgggcactggacgccctgatgaccatttgcccgttaaaggatcagagcgttgaaaagggcattaaattcctgctgaatccgaacctgacagagcaacagacacactatccgacaggcattggtgcaccgggccagttctatattcagtaccacagctacaatgatatctttcctttactggccctggcccactacgcaaaaaagcatagtagctaa

SEQ ID NO: 12 - DNA, 1878 bp, Bacillus megaterium
gtgattattctgctgaaagaggttcagctggagatccagcgtcgcatcgcctatttacgcccgacccagaaaaatgacggcagtttccgctactgcttcgagaccggcgtgatgccggacgcctttctgattatgctgctgcgtaccttcgacctggacaaagaagttctgattaagcagttaaccgagcgcattgtgagcctgcagaacgaagatggtctgtggacactgtttgacgatgaggagcacaacctgagtgccacaatccaggcctataccgccctgctgtacagcggctattaccagaaaaatgaccgcatcttacgtaaggccgaacgctacattatcgatagcggcggcatcagccgtgcacatttcctgacccgttggatgctgagcgttaatggcctgtacgaatggccgaagctgttctacctgccgttaagcctgctgctggttccgacctacgtgccgctgaacttttatgagctgagcacctatgcccgtattcactttgttccgatgatggtggccggtaataaaaaattcagcttaaccagccgccatacccctagtctgagccacctggatgtgcgtgaacaaaaacaggagagtgaagaaaccacccaggagagccgcgcaagcatcttcttagtggatcatctgaaacagctggccagcctgccgagttacattcataagctgggctaccaggcagcagaacgctatatgctggaacgcatcgaaaaggacggcacactgtacagttacgccaccagcaccttttttatgatttacggcctgctggccctgggctacaaaaaggatagctttgtgattcagaaagcaattgatggcatttgtagtctgctgagtacatgcagcggtcacgtgcacgttgaaaacagtaccagcaccgtttgggacaccgcactgctgagctatgccctgcaagaagcaggcgtgccgcagcaggacccgatgattaagggtaccacccgttatctgaagaaacgccagcatacaaaactgggcgactggcagtttcacaatccgaacaccgcaccgggcggttggggctttagcgacattaacaccaacaatcctgatctggatgataccagcgccgcaattcgtgcattaagccgccgcgcccagaccgacacagattacctggaaagctggcagcgcggcatcaattggctgctgagcatgcagaacaaggacggcggctttgccgcatttgaaaagaacaccgatagtatcctgttcacctacctgcctctggaaaatgcaaaggatgccgcaaccgatccggccaccgccgatttaaccggccgcgttttagaatgcctgggtaacttcgccggcatgaacaaaagccatccgagcattaaagccgccgtgaaatggctgttcgaccaccagctggataacggtagctggtacggtcgttggggcgtgtgctatatttacggcacctgggccgcaatcacaggtctgcgcgccgtgggtgttagtgccagcgatccgcgtatcatcaaggcaatcaactggctgaaaagcattcagcaagaagatggtggctttggcgaaagctgctacagcgccagcctgaaaaagtatgttccgctgagtttcagcaccccgagtcagacagcctgggcactggacgccctgatgaccatttgcccgttaaaggatcagagcgttgaaaagggcattaaattcctgctgaatccgaacctgacagagcaacagacacactatccgacaggcattggttttccgggccagttctatattcagtaccacagctacaatgatatctttcctttactggccctggcccactacgcaaaaaagcatagtagctaa

SEQ ID NO: 13 - protein, 625 aa, Bacillus megaterium
MIILLKEVQLEIQRRIAYLRPTQKNDGSFRYCFETGVMPDAFLIMLLRTFDLDKEVLIKQLTERIVSLQNEDGLWTLFDDEEHNLSATIQAYTALLYSGYYQKNDRILRKAERYIIDSGGISRAHFLTRWMLSVNGLYEWPKLFYLPLSLLLVPTYVPLNFYELSTYARIHFVPMMVAGNKKFSLTSRHTPSLSHLDVREQKQESEETTQESRASIFLVDHLKQLASLPSYIHKLGYQAAERYMLERIEKDGTLYSYATSTFFMIYGLLALGYKKDSFVIQKAIDGICSLLSTCSGHVHVENSTSTVWDTALLSYALQEAGVPQQDPMIKGTTRYLKKRQHTKLGDWQFHNPNTAPGGWGFSDINTNNPDLDDTSAAIRALSRRAQTDTDYLESWQRGINWLLSMQNKDGGFAAFEKNTDSILFTYLPLENAKDAATDPATADLTGRVLECLGNFAGMNKSHPSIKAAVKWLFDHQLDNGSWYGRWGVCYIYGTWAAITGLRAVGVSASDPRIIKAINWLKSIQQEDGGFGESCYSASLKKYVPLSFSTPSQTAWALDALMTICPLKDQSVEKGIKFLLNPNLTEQQTHYPTGIGVPGQFYIQYHSYNDIFPLLALAHYAKKHSS

SEQ ID NO: 14 - DNA, 1878 bp, Bacillus megaterium
gtgattattctgctgaaagaggttcagctggagatccagcgtcgcatcgcctatttacgcccgacccagaaaaatgacggcagtttccgctactgcttcgagaccggcgtgatgccggacgcctttctgattatgctgctgcgtaccttcgacctggacaaagaagttctgattaagcagttaaccgagcgcattgtgagcctgcagaacgaagatggtctgtggacactgtttgacgatgaggagcacaacctgagtgccacaatccaggcctataccgccctgctgtacagcggctattaccagaaaaatgaccgcatcttacgtaaggccgaacgctacattatcgatagcggcggcatcagccgtgcacatttcctgacccgttggatgctgagcgttaatggcctgtacgaatggccgaagctgttctacctgccgttaagcctgctgctggttccgacctacgtgccgctgaacttttatgagctgagcacctatgcccgtattcactttgttccgatgatggtggccggtaataaaaaattcagcttaaccagccgccatacccctagtctgagccacctggatgtgcgtgaacaaaaacaggagagtgaagaaaccacccaggagagccgcgcaagcatcttcttagtggatcatctgaaacagctggccagcctgccgagttacattcataagctgggctaccaggcagcagaacgctatatgctggaacgcatcgaaaaggacggcacactgtacagttacgccaccagcaccttttttatgatttacggcctgctggccctgggctacaaaaaggatagctttgtgattcagaaagcaattgatggcatttgtagtctgctgagtacatgcagcggtcacgtgcacgttgaaaacagtaccagcaccgtttgggacaccgcactgctgagctatgccctgcaagaagcaggcgtgccgcagcaggacccgatgattaagggtaccacccgttatctgaagaaacgccagcatacaaaactgggcgactggcagtttcacaatccgaacaccgcaccgggcggttggggctttagcgacattaacaccaacaatcctgatctggatgataccagcgccgcaattcgtgcattaagccgccgcgcccagaccgacacagattacctggaaagctggcagcgcggcatcaattggctgctgagcatgcagaacaaggacggcggctttgccgcatttgaaaagaacaccgatagtatcctgttcacctacctgcctctggaaaatgcaaaggatgccgcaaccgatccggccaccgccgatttaaccggccgcgttttagaatgcctgggtaacttcgccggcatgaacaaaagccatccgagcattaaagccgccgtgaaatggctgttcgaccaccagctggataacggtagctggtacggtcgttggggcgtgtgctatatttacggcacctgggccgcaatcacaggtctgcgcgccgtgggtgttagtgccagcgatccgcgtatcatcaaggcaatcaactggctgaaaagcattcagcaagaagatggtggctttggcgaaagctgctacagcgccagcctgaaaaagtatgttccgctgagtttcagcaccccgagtcagacagcctgggcactggacgccctgatgaccatttgcccgttaaaggatcagagcgttgaaaagggcattaaattcctgctgaatccgaacctgacagagcaacagacacactatccgacaggcattggtgttccgggccagttctatattcagtaccacagctacaatgatatctttcctttactggccctggcccactacgcaaaaaagcatagtagctaa